European Patent Application EP 4 520 833 A1, published March 12, 2025. Title: Virus-derived construct plasmid. Applicant: Synplogen Co., Ltd. Application JP. The sequence listing filed with the application follows.

SEQUENCE LISTING (188 sequences)

SEQ ID NO: 1 - DNA, 21 bp, synthetic construct
  misc_feature 1..21: note = primer
  source 1..21: mol_type = other DNA
ggaacccctagtgatggagtt

SEQ ID NO: 2 - DNA, 16 bp, synthetic construct
  misc_feature 1..16: note = primer
  source 1..16: mol_type = other DNA
cggcctcagtgagcga

SEQ ID NO: 3 - DNA, 27 bp, synthetic construct
  misc_feature 1..27: note = linker(F)
  source 1..27: mol_type = other DNA
agcttgcgcaggtgcacctgcatgcgg

SEQ ID NO: 4 - DNA, 27 bp, synthetic construct
  misc_feature 1..27: note = linker(R)
  source 1..27: mol_type = other DNA
agctccgcatgcaggtgcacctgcgca

SEQ ID NO: 5 - DNA, 180 bp, synthetic construct
  misc_feature 1..180: note = segment 1-1
  source 1..180: mol_type = other DNA
tagaggcaagggttgtttttattgactacacctgcgatcaagcttgcctgcaggcagctgcgcgctcgctcgctcactgaggccgcccgggcaaagcccgggcgtcgggcgacctttggtcgcccggcctcagtgagcgagcgagcgcgcagagagggagtggccaactccatcactagg

SEQ ID NO: 6 - DNA, 155 bp, synthetic construct
  misc_feature 1..155: note = segment 1-2
  source 1..155: mol_type = other DNA
ggtcgttgggcggtcagccaggcgggccatttaccgtaagttatgtaacgcggaactccatatatgggctatgaactaatgaccccgtaattgattactattaaagcttgatatcgataggaacccctagtgatggagttggccactccctctct

SEQ ID NO: 7 - DNA, 155 bp, synthetic construct
  misc_feature 1..155: note = segment 1-3
  source 1..155: mol_type = other DNA
atggcccgcctggctgaccgcccaacgacccccgcccattgacgtcaataatgacgtatgttcccatagtaacgccaatagggactttccattgacgtcaatgggtggagtatttacggtaaactgcccacttggcagtacatcaagtgtatcat

SEQ ID NO: 8 - DNA, 155 bp, synthetic construct
  misc_feature 1..155: note = segment 1-4
  source 1..155: mol_type = other DNA
gtaatagcgatgactaatacgtagatgtactgccaagtaggaaagtcccataaggtcatgtactgggcataatgccaggcgggccatttaccgtcattgacgtcaatagggggcgtacttggcatatgatacacttgatgtactgccaagtgggc

SEQ ID NO: 9 - DNA, 155 bp, synthetic construct
  misc_feature 1..155: note = segment 1-5
  source 1..155: mol_type = other DNA
gtacatctacgtattagtcatcgctattaccatggtgatgcggttttggcagtacatcaatgggcgtggatagcggtttgactcacggggatttccaagtctccaccccattgacgtcaatgggagtttgttttggcaccaaaatcaacgggact

SEQ ID NO: 10 - DNA, 177 bp, synthetic construct
  misc_feature 1..177: note = segment 1-6
  source 1..177: mol_type = other DNA
tactggttggaagaaagacctctatcacctgcgatcctgggcccttaaggatatccactaaaccagctctgcttatatagacctcccaccgtacacgcctaccgcccatttgcgtcaatggggcggagttgttacgacattttggaaagtcccgttgattttggtgccaaaacaaac

SEQ ID NO: 11 - DNA, 177 bp, synthetic construct
  misc_feature 1..177: note = segment 3-1
  source 1..177: mol_type = other DNA
tagaggcaagggttgtttttattgactacacctgcgatcggaaccaagctggagtgcagtggcacaatcttggctcactgcaatctccgcctcctgggttcaagcgattctcctgcctcagcctcccgagttgttgggattccaggcatgcatgaccaggctcagctaatttttgtt

SEQ ID NO: 12 - DNA, 150 bp, synthetic construct
  misc_feature 1..150: note = segment 3-2
  source 1..150: mol_type = other DNA
agggagcagtggttcacgcctgtaatcccagcaatttgggaggccaaggtgggtagatcacctgagattaggagttggagaccagcctggccaatatggtgaaaccccgtctctaccaaaaaaacaaaaattagctgagcctggtcatgc

SEQ ID NO: 13 - DNA, 152 bp, synthetic construct
  misc_feature 1..152: note = segment 3-3
  source 1..152: mol_type = other DNA
ggattacaggcgtgaaccactgctcccttccctgtccttatcgatagatctaggaacccctagtgatggagttggccactccctctctgcgcgctcgctcgctcactgaggccgggcgaccaaaggtcgcccgacgcccgggctttgcccgg

SEQ ID NO: 14 - DNA, 152 bp, synthetic construct
  misc_feature 1..152: note = segment 3-4
  source 1..152: mol_type = other DNA
ggaagctgtagagctgttcctggttgcgacgcagggtgggctgtacctggggactgttaagcatggagttgggtaccggatctgcctgcaggcagctgcgcgctcgctcgctcactgaggccgcccgggcaaagcccgggcgtcgggcgacc

SEQ ID NO: 15 - DNA, 151 bp, synthetic construct
  misc_feature 1..151: note = segment 3-5
  source 1..151: mol_type = other DNA
cgcaaccaggaacagctctacagcttcctggagcgccactcgccctacttccgcagccacagtgcgcagattaggagcgccacttctttttgtcacttgaaaaacatgtaaaaataatgtactaggagacactttcaataaaggcaaatgt

SEQ ID NO: 16 - DNA, 174 bp, synthetic construct
  misc_feature 1..174: note = segment 3-6
  source 1..174: mol_type = other DNA
tactggttggaagaaagacctctatcacctgcgatctgtccctgccagtggcgcatagcgatgcgcggcagaacccctttgatttttaaacggcgcagacggcaagggtggggggtaaataatcacccgagagtgtacaaataaaaacatttgcctttattgaaagtgtctcct

SEQ ID NO: 17 - DNA, 179 bp, synthetic construct
  misc_feature 1..179: note = segment 16-1
  source 1..179: mol_type = other DNA
tagaggcaagggttgtttttattgactaggtctcgcaggtacatctacggattacgtcgacgtttaaaccatatgagcggccgctctagaactagtggatcccccggaagatcagaagttcctattccgaagttcctattctctagaaagtataggaacttctgatctgcgcagccgcc

SEQ ID NO: 18 - DNA, 154 bp, synthetic construct
  misc_feature 1..154: note = segment 16-2
  source 1..154: mol_type = other DNA
cagaatctggcggcaactcccattccttctcggccacccagttcacaaagctgtcagaaatgccgggcagatgctcgtcaaggtcgctggggaccttaatcacaatctcgtaaaaccccggcatggcggctgcgcagatcagaagttcctatac

SEQ ID NO: 19 - DNA, 150 bp, synthetic construct
  misc_feature 1..150: note = segment 16-3
  source 1..150: mol_type = other DNA
agaaggaatgggagttgccgccagattctgacatggatctgaatctgattgagcaggcacccctgaccgtggccgagaagctgcagcgcgactttctgacggaatggcgccgtgtgagtaaggccccggaggcccttttctttgtgcaat

SEQ ID NO: 20 - DNA, 154 bp, synthetic construct
  misc_feature 1..154: note = segment 16-4
  source 1..154: mol_type = other DNA
ccgcggtaaattctctgaatcagtttttcgcgaatctgactcaggaaacgtcccaaaaccatggatttcaccccggtggtttccacgagcacgtgcatgtggaagtagctctctcccttctcaaattgcacaaagaaaagggcctccggggcct

SEQ ID NO: 21 - DNA, 154 bp, synthetic construct
  misc_feature 1..154: note = segment 16-5
  source 1..154: mol_type = other DNA
cgaaaaactgattcagagaatttaccgcgggatcgagccgactttgccaaactggttcgcggtcacaaagaccagaaatggcgccggaggcgggaacaaggtggtggatgagtgctacatccccaattacttgctccccaaaacccagcctgag

SEQ ID NO: 22 - DNA, 176 bp, synthetic construct
  misc_feature 1..176: note = segment 16-6
  source 1..176: mol_type = other DNA
tactggttggaagaaagacctctatggtctccctgctcctgcgtctgcgacacgtgcgtcagatgctgcgccaccaaccgtttacgctccgtgagattcaaacaggcgcttaaatactgttccatattagtccacgcccactggagctcaggctgggttttggggagcaagtaatt

SEQ ID NO: 23 - DNA, 31 bp, synthetic construct
  misc_feature 1..31: note = primer 1-F
  source 1..31: mol_type = other DNA
tagcacctgcatgcaagcttgcctgcaggca

SEQ ID NO: 24 - DNA, 33 bp, synthetic construct
  misc_feature 1..33: note = primer 1-R
  source 1..33: mol_type = other DNA
tagcacctgcgcatctgggcccttaaggatatc

SEQ ID NO: 25 - DNA, 20 bp, synthetic construct
  misc_feature 1..20: note = primer 2-F
  source 1..20: mol_type = other DNA
tagggtctcgccagccggcc

SEQ ID NO: 26 - DNA, 28 bp, synthetic construct
  misc_feature 1..28: note = primer 2-R
  source 1..28: mol_type = other DNA
tagggtctccttcccaatagaccccgca

SEQ ID NO: 27 - DNA, 31 bp, synthetic construct
  misc_feature 1..31: note = primer 3-F
  source 1..31: mol_type = other DNA
tagcacctgcatgcggaaccaagctggagtg

SEQ ID NO: 28 - DNA, 29 bp, synthetic construct
  misc_feature 1..29: note = primer 3-R
  source 1..29: mol_type = other DNA
tagcacctgcgcattgtccctgccagtgg

SEQ ID NO: 29 - DNA, 29 bp, synthetic construct
  misc_feature 1..29: note = primer 4-F
  source 1..29: mol_type = other DNA
tagggtctcggacacgttgcgatactggt

SEQ ID NO: 30 - DNA, 23 bp, synthetic construct
  misc_feature 1..23: note = primer 4-R
  source 1..23: mol_type = other DNA
tagggtctcccacgagcccacgg

SEQ ID NO: 31 - DNA, 33 bp, synthetic construct
  misc_feature 1..33: note = primer 5-F
  source 1..33: mol_type = other DNA
tagcacctgcatgccgtggtgcttgtaggttac

SEQ ID NO: 32 - DNA, 26 bp, synthetic construct
  misc_feature 1..26: note = primer 5-R
  source 1..26: mol_type = other DNA
tagcacctgcgcatgagcgcggacgc

SEQ ID NO: 33 - DNA, 23 bp, synthetic construct
  misc_feature 1..23: note = primer 6-F
  source 1..23: mol_type = other DNA
tagggtctcggctcgggggtggt

SEQ ID NO: 34 - DNA, 26 bp, synthetic construct
  misc_feature 1..26: note = primer 6-R
  source 1..26: mol_type = other DNA
tagggtctccttgccgcgcgtttctc

SEQ ID NO: 35 - DNA, 34 bp, synthetic construct
  misc_feature 1..34: note = primer 7-F
  source 1..34: mol_type = other DNA
tagcacctgcatgcgcaaacgctctgcaacaaga

SEQ ID NO: 36 - DNA, 27 bp, synthetic construct
  misc_feature 1..27: note = primer 7-R
  source 1..27: mol_type = other DNA
tagcacctgcgcatgtccgccaggtgc

SEQ ID NO: 37 - DNA, 30 bp, synthetic construct
  misc_feature 1..30: note = primer 8-F
  source 1..30: mol_type = other DNA
tagggtctcgggacattatcttccccgaac

SEQ ID NO: 38 - DNA, 21 bp, synthetic construct
  misc_feature 1..21: note = primer 8-R
  source 1..21: mol_type = other DNA
tagggtctccgtggcggcggc

SEQ ID NO: 39 - DNA, 28 bp, synthetic construct
  misc_feature 1..28: note = primer 9-F
  source 1..28: mol_type = other DNA
tagcacctgcatgcccacccacggacga

SEQ ID NO: 40 - DNA, 29 bp, synthetic construct
  misc_feature 1..29: note = primer 9-R
  source 1..29: mol_type = other DNA
tagcacctgcgcatgagggagcgcagaga

SEQ ID NO: 41 - DNA, 25 bp, synthetic construct
  misc_feature 1..25: note = primer 10-F
  source 1..25: mol_type = other DNA
tagggtctcgcctcacccgcagctg

SEQ ID NO: 42 - DNA, 39 bp, synthetic construct
  misc_feature 1..39: note = primer 10-R
  source 1..39: mol_type = other DNA
tagggtctccgactaaaaaatgacgtaacggttaaagtc

SEQ ID NO: 43 - DNA, 40 bp, synthetic construct
  misc_feature 1..40: note = primer 11-F
  source 1..40: mol_type = other DNA
tagcacctgcatgcagtcctatatatactcgctctgtact

SEQ ID NO: 44 - DNA, 32 bp, synthetic construct
  misc_feature 1..32: note = primer 11-R
  source 1..32: mol_type = other DNA
tagcacctgcgcatggagctatgctaaccagc

SEQ ID NO: 45 - DNA, 28 bp, synthetic construct
  misc_feature 1..28: note = primer 12-F
  source 1..28: mol_type = other DNA
tagggtctcgctccgagtatgcgtgtca

SEQ ID NO: 46 - DNA, 36 bp, synthetic construct
  misc_feature 1..36: note = primer 12-R
  source 1..36: mol_type = other DNA
tagggtctccgtagttgtagtatatccactctctca

SEQ ID NO: 47 - DNA, 33 bp, synthetic construct
  misc_feature 1..33: note = primer 13-F
  source 1..33: mol_type = other DNA
tagcacctgcatgcctactacacagagcgagct

SEQ ID NO: 48 - DNA, 37 bp, synthetic construct
  misc_feature 1..37: note = primer 13-R
  source 1..37: mol_type = other DNA
tagcacctgcgcatgcacagcaccacaatattgttca

SEQ ID NO: 49 - DNA, 33 bp, synthetic construct
  misc_feature 1..33: note = primer 14-F
  source 1..33: mol_type = other DNA
tagcacctgcatgcgtgctgcagttactgtgct

SEQ ID NO: 50 - DNA, 36 bp, synthetic construct
  misc_feature 1..36: note = primer 14-R
  source 1..36: mol_type = other DNA
tagcacctgcgcattagcgaggtaagcacttactct

SEQ ID NO: 51 - DNA, 34 bp, synthetic construct
  misc_feature 1..34: note = primer 15-F
  source 1..34: mol_type = other DNA
tagggtctcggctagtttctgtggattcactaga

SEQ ID NO: 52 - DNA, 27 bp, synthetic construct
  misc_feature 1..27: note = primer 15-R
  source 1..27: mol_type = other DNA
tagggtctcccctggacatccaggtga

SEQ ID NO: 53 - DNA, 32 bp, synthetic construct
  misc_feature 1..32: note = primer 16-F
  source 1..32: mol_type = other DNA
tagggtctcgcaggtacatctacggattacgt

SEQ ID NO: 54 - DNA, 25 bp, synthetic construct
  misc_feature 1..25: note = primer 16-R
  source 1..25: mol_type = other DNA
tagggtctccctgctcctgcgtctg

SEQ ID NO: 55 - DNA, 38 bp, synthetic construct
  misc_feature 1..38: note = primer 17-F
  source 1..38: mol_type = other DNA
tagcacctgcatgcgcagaacaaagagaatcagaatcc

SEQ ID NO: 56 - DNA, 38 bp, synthetic construct
  misc_feature 1..38: note = primer 17-R
  source 1..38: mol_type = other DNA
tagcacctgcgcatggtgagttcaaatttgaacatccg

SEQ ID NO: 57 - DNA, 23 bp, synthetic construct
  misc_feature 1..23: note = primer 18-F
  source 1..23: mol_type = other DNA
tagggtctcgcacccgccgtctg

SEQ ID NO: 58 - DNA, 21 bp, synthetic construct
  misc_feature 1..21: note = primer 18-R
  source 1..21: mol_type = other DNA
tagggtctcccgagggccgcg

SEQ ID NO: 59 - DNA, 31 bp, synthetic construct
  misc_feature 1..31: note = primer 19-F
  source 1..31: mol_type = other DNA
tagcacctgcatgcctcgagcacgacaaagc

SEQ ID NO: 60 - DNA, 44 bp, synthetic construct
  misc_feature 1..44: note = primer 19-R
  source 1..44: mol_type = other DNA
tagcacctgcgcattgacttgaatgttaaagagcttgaagttga

SEQ ID NO: 61 - DNA, 29 bp, synthetic construct
  misc_feature 1..29: note = primer 20-F
  source 1..29: mol_type = other DNA
tagggtctcggtcaaagaggtcacgcaga

SEQ ID NO: 62 - DNA, 33 bp, synthetic construct
  misc_feature 1..33: note = primer 20-R
  source 1..33: mol_type = other DNA
tagggtctccttggttgtcctgatttcctcttc

SEQ ID NO: 63 - DNA, 30 bp, synthetic construct
  misc_feature 1..30: note = primer 21-F
  source 1..30: mol_type = other DNA
tagcacctgcatgcccaatcccgtggctac

SEQ ID NO: 64 - DNA, 39 bp, synthetic construct
  misc_feature 1..39: note = primer 21-R
  source 1..39: mol_type = other DNA
tagcacctgcgcatgcatatgatacacttgatgtactgc

SEQ ID NO: 65 - DNA, 28 bp, synthetic construct
  misc_feature 1..28: note = primer 22-F
  source 1..28: mol_type = other DNA
tagggtctcgatgccaagtacgccccct

SEQ ID NO: 66 - DNA, 25 bp, synthetic construct
  misc_feature 1..25: note = primer 22-R
  source 1..25: mol_type = other DNA
tagggtctccctcccgggctgtagt

SEQ ID NO: 67 - DNA, 870 bp, synthetic construct
  misc_feature 1..870: note = fragment 1
  source 1..870: mol_type = other DNA
tagaggcaagggttgtttttattgactacacctgcgatcaaaagtgccacctgacgtctaagaaaccattattatcatgacattaacctataaaaataggcgtatcacgaggccctttcgtcttcaagaattctcatgtttgacagcttatcatcgataagcttgcctgcaggcagctgcgcgctcgctcgctcactgaggccgcccgggcaaagcccgggcgtcgggcgacctttggtcgcccggcctcagtgagcgagcgagcgcgcagagagggagtggccaactccatcactaggggttcctatcgatatcaagctttaatagtaatcaattacggggtcattagttcatagcccatatatggagttccgcgttacataacttacggtaaatggcccgcctggctgaccgcccaacgacccccgcccattgacgtcaataatgacgtatgttcccatagtaacgccaatagggactttccattgacgtcaatgggtggagtatttacggtaaactgcccacttggcagtacatcaagtgtatcatatgccaagtacgccccctattgacgtcaatgacggtaaatggcccgcctggcattatgcccagtacatgaccttatgggactttcctacttggcagtacatctacgtattagtcatcgctattaccatggtgatgcggttttggcagtacatcaatgggcgtggatagcggtttgactcacggggatttccaagtctccaccccattgacgtcaatgggagtttgttttggcaccaaaatcaacgggactttccaaaatgtcgtaacaactccgccccattgacggatcgcaggtgatagaggtctttcttccaaccagta

SEQ ID NO: 68 - DNA, 865 bp, synthetic construct
  misc_feature 1..865: note = fragment 2
  source 1..865: mol_type = other DNA
tagaggcaagggttgtttttattgactagaagacgagacgcaaatgggcggtaggcgtgtacggtgggaggtctatataagcagagctggtttagtggatatcgtatacgccaccatggtgagcaagggcgaggagctgttcaccggggtggtgcccatcctggtcgagctggacggcgacgtaaacggccacaagttcagcgtgtccggcgagggcgagggcgatgccacctacggcaagctgaccctgaagttcatctgcaccaccggcaagctgcccgtgccctggcccaccctcgtgaccaccctgacctacggcgtgcagtgcttcagccgctaccccgaccacatgaagcagcacgacttcttcaagtccgccatgcccgaaggctacgtccaggagcgcaccatcttcttcaaggacgacggcaactacaagacccgcgccgaggtgaagttcgagggcgacaccctggtgaaccgcatcgagctgaagggcatcgacttcaaggaggacggcaacatcctggggcacaagctggagtacaactacaacagccacaacgtctatatcatggccgacaagcagaagaacggcatcaaggtgaacttcaagatccgccacaacatcgaggacggcagcgtgcagctcgccgaccactaccagcagaacacccccatcggcgacggccccgtgctgctgcccgacaaccactacctgagcacccagtccgccctgagcaaagaccccaacgagaagcgcgatcacatggtcctgctggagttcgtgaccgccgccgggatcactctcggcatggacgagctgtacaaggagtcttcatagaggtctttcttccaaccagta

SEQ ID NO: 69 - DNA, 872 bp, synthetic construct
  misc_feature 1..872: note = fragment 3
  source 1..872: mol_type = other DNA
tagaggcaagggttgtttttattgactacacctgcgatccaagtaagtataccgataatcaacctctggattacaaaatttgtgaaagattgactggtattcttaactatgttgctccttttacgctatgtggatacgctgctttaatgcctttgtatcatgctattgcttcccgtatggctttcattttctcctccttgtataaatcctggttgctgtctctttatgaggagttgtggcccgttgtcaggcaacgtggcgtggtgtgcactgtgtttgctgacgcaacccccactggttggggcattgccaccacctgtcagctcctttccgggactttcgctttccccctccctattgccacggcggaactcatcgccgcctgccttgcccgctgctggacaggggctcggctgttgggcactgacaattccgtggtgttgtcggggaagctgacgtcctttccatggctgctcgcctgtgttgccacctggattctgcgcgggacgtccttctgctacgtcccttcggccctcaatccagcggaccttccttcccgcggcctgctgccggctctgcggcctcttccgcgtcttcgccttcgccctcagacgagtcggatctccctttgggccgcctccccgcatcggttaattaaacgggtggcatccctgtgacccctccccagtgcctctcctggccctggaagttgccactccagtgcccaccagccttgtcctaataaaattaagttgcatcattttgtctgactaggtgtccttctataatattatggggtggaggggggtggtatggagcaaggggcaagttgggaagatcgcaggtgatagaggtctttcttccaaccagta

SEQ ID NO: 70 - DNA, 874 bp, synthetic construct
  misc_feature 1..874: note = fragment 4
  source 1..874: mol_type = other DNA
tagaggcaagggttgtttttattgactacacctgcgatcggaagacaacctgtagggcctgcggggtctattgggaaccaagctggagtgcagtggcacaatcttggctcactgcaatctccgcctcctgggttcaagcgattctcctgcctcagcctcccgagttgttgggattccaggcatgcatgaccaggctcagctaatttttgtttttttggtagagacggggtttcaccatattggccaggctggtctccaactcctaatctcaggtgatctacccaccttggcctcccaaattgctgggattacaggcgtgaaccactgctcccttccctgtccttatcgatagatctaggaacccctagtgatggagttggccactccctctctgcgcgctcgctcgctcactgaggccgggcgaccaaaggtcgcccgacgcccgggctttgcccgggcggcctcagtgagcgagcgagcgcgcagctgcctgcaggcagatcccctcgaggggtacccaactccatgcttaacagtccccaggtacagcccaccctgcgtcgcaaccaggaacagctctacagcttcctggagcgccactcgccctacttccgcagccacagtgcgcagattaggagcgccacttctttttgtcacttgaaaaacatgtaaaaataatgtactaggagacactttcaataaaggcaaatgtttttatttgtacactctcgggtgattatttaccccccacccttgccgtctgcgccgtttaaaaatcaaaggggttctgccgcgcatcgctatgcgccactggcagggacacgttgcgatactggtggatcgcaggtgatagaggtctttcttccaaccagta

SEQ ID NO: 71 - DNA, 866 bp, synthetic construct
  misc_feature 1..866: note = fragment 5
  source 1..866: mol_type = other DNA
tagaggcaagggttgtttttattgactagaagacgaggtgtttagtgctccacttaaactcaggcacaaccatccgcggcagctcggtgaagttttcactccacaggctgcgcaccatcaccaacgcgtttagcaggtcgggcgccgatatcttgaagtcgcagttggggcctccgccctgcgcgcgcgagttgcgatacacagggttgcagcactggaacactatcagcgccgggtggtgcacgctggccagcacgctcttgtcggagatcagatccgcgtccaggtcctccgcgttgctcagggcgaacggagtcaactttggtagctgccttcccaaaaagggtgcatgcccaggctttgagttgcactcgcaccgtagtggcatcagaaggtgaccgtgcccggtctgggcgttaggatacagcgcctgcatgaaagccttgatctgcttaaaagccacctgagcctttgcgccttcagagaagaacatgccgcaagacttgccggaaaactgattggccggacaggccgcgtcatgcacgcagcaccttgcgtcggtgttggagatctgcaccacatttcggccccaccggttcttcacgatcttggccttgctagactgctccttcagcgcgcgctgcccgttttcgctcgtcacatccatttcaatcacgtgctccttatttatcataatgctcccgtgtagacacttaagctcgccttcgatctcagcgcagcggtgcagccacaacgcgcagcccgtgggctcgtggtgcttgtaggttacctctgcaaacgactgcaggtacgcctgcaggaatcgccccatcgagtcttcatagaggtctttcttccaaccagta

SEQ ID NO: 72 - DNA, 865 bp, synthetic construct
  misc_feature 1..865: note = fragment 6
  source 1..865: mol_type = other DNA
tagaggcaagggttgtttttattgactacacctgcgatccatcatcgtcacaaaggtcttgttgctggtgaaggtcagctgcaacccgcggtgctcctcgtttagccaggtcttgcatacggccgccagagcttccacttggtcaggcagtagcttgaagtttgcctttagatcgttatccacgtggtacttgtccatcaacgcgcgcgcagcctccatgcccttctcccacgcagacacgatcggcaggctcagcgggtttatcaccgtgctttcactttccgcttcactggactcttccttttcctcttgcgtccgcataccccgcgccactgggtcgtcttcattcagccgccgcaccgtgcgcttacctcccttgccgtgcttgattagcaccggtgggttgctgaaacccaccatttgtagcgccacatcttctctttcttcctcgctgtccacgatcacctctggggatggcgggcgctcgggcttgggagaggggcgcttctttttctttttggacgcaatggccaaatccgccgtcgaggtcgatggccgcgggctgggtgtgcgcggcaccagcgcatcttgtgacgagtcttcttcgtcctcggactcgagacgccgcctcagccgcttttttgggggcgcgcggggaggcggcggcgacggcgacggggacgacacgtcctccatggttggtggacgtcgcgccgcaccgcgtccgcgctcgggggtggtttcgcgctgctcctcttcccgactggccatttccttctcctataggcagaaaaagatcatggagtcagtcgagaaggaggacagcctagatcgcaggtgatagaggtctttcttccaaccagta

SEQ ID NO: 73 - DNA, 873 bp, synthetic construct
  misc_feature 1..873: note = fragment 7
  source 1..873: mol_type = other DNA
tagaggcaagggttgtttttattgactacacctgcgatccctaaccgccccctttgagttcgccaccaccgcctccaccgatgccgccaacgcgcctaccaccttccccgtcgaggcacccccgcttgaggaggaggaagtgattatcgagcaggacccaggttttgtaagcgaagacgacgaggatcgctcagtaccaacagaggataaaaagcaagaccaggacgacgcagaggcaaacgaggaacaagtcgggcggggggaccaaaggcatggcgactacctagatgtgggagacgacgtgctgttgaagcatctgcagcgccagtgcgccattatctgcgacgcgttgcaagagcgcagcgatgtgcccctcgccatagcggatgtcagccttgcctacgaacgccacctgttctcaccgcgcgtaccccccaaacgccaagaaaacggcacatgcgagcccaacccgcgcctcaacttctaccccgtatttgccgtgccagaggtgcttgccacctatcacatctttttccaaaactgcaagatacccctatcctgccgtgccaaccgcagccgagcggacaagcagctggccttgcggcagggcgctgtcatacctgatatcgcctcgctcgacgaagtgccaaaaatctttgagggtcttggacgcgacgagaaacgcgcggcaaacgctctgcaacaagaaaacagcgaaaatgaaagtcactgtggagtgctggtggaacttgagggtgacaacgcgcgcctagccgtgctgaaacgcagcatcgaggtcacccactttgcctacccggcacttaacctaccccccaagatcgcaggtgatagaggtctttcttccaaccagta

SEQ ID NO: 74 - DNA, 870 bp, synthetic construct
  misc_feature 1..870: note = fragment 8
  source 1..870: mol_type = other DNA
tagaggcaagggttgtttttattgactagaagacgaccaaggttatgagcacagtcatgagcgagctgatcgtgcgccgtgcacgacccctggagagggatgcaaacttgcaagaacaaaccgaggagggcctacccgcagttggcgatgagcagctggcgcgctggcttgagacgcgcgagcctgccgacttggaggagcgacgcaagctaatgatggccgcagtgcttgttaccgtggagcttgagtgcatgcagcggttctttgctgacccggagatgcagcgcaagctagaggaaacgttgcactacacctttcgccagggctacgtgcgccaggcctgcaaaatttccaacgtggagctctgcaacctggtctcctaccttggaattttgcacgaaaaccgcctcgggcaaaacgtgcttcattccacgctcaagggcgaggcgcgccgcgactacgtccgcgactgcgtttacttatttctgtgctacacctggcaaacggccatgggcgtgtggcagcaatgcctggaggagcgcaacctaaaggagctgcagaagctgctaaagcaaaacttgaaggacctatggacggccttcaacgagcgctccgtggccgcgcacctggcggacattatcttccccgaacgcctgcttaaaaccctgcaacagggtctgccagacttcaccagtcaaagcatgttgcaaaactttaggaactttatcctagagcgttcaggaattctgcccgccacctgctgtgcgcttcctagcgactttgtgcccattaagtaccgtgaatgccctccgccgctttggggtcactgctaccttcgagtcttcatagaggtctttcttccaaccagta

SEQ ID NO: 75 - DNA, 867 bp, synthetic construct
  misc_feature 1..867: note = fragment 9
  source 1..867: mol_type = other DNA
tagaggcaagggttgtttttattgactacacctgcgatccttctgcagctagccaactaccttgcctaccactccgacatcatggaagacgtgagcggtgacggcctactggagtgtcactgtcgctgcaacctatgcaccccgcaccgctccctggtctgcaattcgcaactgcttagcgaaagtcaaattatcggtacctttgagctgcagggtccctcgcctgacgaaaagtccgcggctccggggttgaaactcactccggggctgtggacgtcggcttaccttcgcaaatttgtacctgaggactaccacgcccacgagattaggttctacgaagaccaatcccgcccgccaaatgcggagcttaccgcctgcgtcattacccagggccacatccttggccaattgcaagccatcaacaaagcccgccaagagtttctgctacgaaagggacggggggtttacctggacccccagtccggcgaggagctcaacccaatccccccgccgccgcagccctatcagcagccgcgggcccttgcttcccaggatggcacccaaaaagaagctgcagctgccgccgccgccacccacggacgaggaggaatactgggacagtcaggcagaggaggttttggacgaggaggaggagatgatggaagactgggacagcctagacgaagcttccgaggccgaagaggtgtcagacgaaacaccgtcaccctcggtcgcattcccctcgccggcgccccagaaattggcaaccgttcccagcatcgctacaacctccgctcctcaggcgccgccggcactgcctgttcgccgaccgatcgcaggtgatagaggtctttcttccaaccagta

SEQ ID NO: 76 - DNA, 876 bp, synthetic construct
  misc_feature 1..876: note = fragment 10
  source 1..876: mol_type = other DNA
tagaggcaagggttgtttttattgactacacctgcgatcgacccaaccgtagatgggacaccactggaaccagggccggtaagtctaagcagccgccgccgttagcccaagagcaacaacagcgccaaggctaccgctcgtggcgcgggcacaagaacgccatagttgcttgcttgcaagactgtgggggcaacatctccttcgcccgccgctttcttctctaccatcacggcgtggccttcccccgtaacatcctgcattactaccgtcatctctacagcccctactgcaccggcggcagcggcagcggcagcaacagcagcggtcacacagaagcaaaggcgaccggatagcaagactctgacaaagcccaagaaatccacagcggcggcagcagcaggaggaggagcgctgcgtctggcgcccaacgaacccgtatcgacccgcgagcttagaaataggatttttcccactctgtatgctatatttcaacaaagcaggggccaagaacaagagctgaaaataaaaaacaggtctctgcgctccctcacccgcagctgcctgtatcacaaaagcgaagatcagcttcggcgcacgctggaagacgcggaggctctcttcagcaaatactgcgcgctgactcttaaggactagtttcgcgccctttctcaaatttaagcgcgaaaactacgtcatctccagcggccacacccggcgccagcacctgtcgtcagcgccattatgagcaaggaaattcccacgccctacatgtggagttaccagccacaaatgggacttgcggctggagctgcccaagactactcaacccgaataaactacgatcgcaggtgatagaggtctttcttccaaccagta

SEQ ID NO: 77 - DNA, 855 bp, synthetic construct
  misc_feature 1..855: note = fragment 11
  source 1..855: mol_type = other DNA
tagaggcaagggttgtttttattgactagaagacgactacatgagcgcgggaccccacatgatatcccgggtcaacggaatccgcgcccaccgaaaccgaattctcctcgaacaggcggctattaccaccacacctcgtaataaccttaatccccgtagttggcccgctgccctggtgtaccaggaaagtcccgctcccaccactgtggtacttcccagagacgcccaggccgaagttcagatgactaactcaggggcgcagcttgcgggcggctttcgtcacagggtgcggtcgcccgggcgttttagggcggagtaacttgcatgtattgggaattgtagtttttttaaaatgggaagtgacgtatcgtgggaaaacggaagtgaagatttgaggaagttgtgggttttttggctttcgtttctgggcgtaggttcgcgtgcggttttctgggtgttttttgtggactttaaccgttacgtcattttttagtcctatatatactcgctctgtacttggccctttttacactgtgactgattgagctggtgccgtgtcgagtggtgttttttaataggtttttttactggtaaggctgactgttatggctgccgctgtggaagcgctgtatgttgttctggagcgggagggtgctattttgcctaggcaggagggtttttcaggtgtttatgtgtttttctctcctattaattttgttatacctcctatgggggctgtaatgttgtctctacgcctgcgggtatgtattcccccgggctatttcggtcgctttttagcactgaccgatgttaaccaacctggagtcttcatagaggtctttcttccaaccagta

SEQ ID NO: 78 - DNA, 874 bp, synthetic construct
  misc_feature 1..874: note = fragment 12
  source 1..874: mol_type = other DNA
tagaggcaagggttgtttttattgactagaagacgacctgatgtgtttaccgagtcttacattatgactccggacatgaccgaggaactgtcggtggtgctttttaatcacggtgaccagtttttttacggtcacgccggcatggccgtagtccgtcttatgcttataagggttgtttttcctgttgtaagacaggcttctaatgtttaaatgtttttttttttgttattttattttgtgtttaatgcaggaacccgcagacatgtttgagagaaaaatggtgtctttttctgtggtggttccggaacttacctgcctttatctgcatgagcatgactacgatgtgcttgcttttttgcgcgaggctttgcctgattttttgagcagcaccttgcattttatatcgccgcccatgcaacaagcttacataggggctacgctggttagcatagctccgagtatgcgtgtcataatcagtgtgggttcttttgtcatggttcctggcggggaagtggccgcgctggtccgtgcagacctgcacgattatgttcagctggccctgcgaagggacctacgggatcgcggtatttttgttaatgttccgcttttgaatcttatacaggtctgtgaggaacctgaatttttgcaatcatgattcgctgcttgaggctgaaggtggagggcgctctggagcagatttttacaatggccggacttaatattcgggatttgcttagagacatattgataaggtggcgagatgaaaattatttgggcatggttgaaggtgctggaatgtttatagaggagattcaccctgaagggtttagcctttacgtccgagtcttcatagaggtctttcttccaaccagta

SEQ ID NO: 79 - DNA, 869 bp, synthetic construct
  misc_feature 1..869: note = fragment 13
  source 1..869: mol_type = other DNA
tagaggcaagggttgtttttattgactacacctgcgatcgtccacttggacgtgagggcagtttgccttttggaagccattgtgcaacatcttacaaatgccattatctgttctttggctgtagagtttgaccacgccaccggaggggagcgcgttcacttaatagatcttcattttgaggttttggataatcttttggaataaaaaaaaaaaaacatggttcttccagctcttcccgctcctcccgtgtgtgactcgcagaacgaatgtgtaggttggctgggtgtggcttattctgcggtggtggatgttatcagggcagcggcgcatgaaggagtttacatagaacccgaagccagggggcgcctggatgctttgagagagtggatatactacaactactacacagagcgagctaagcgacgagaccggagacgcagatctgtttgtcacgcccgcacctggttttgcttcaggaaatatgactacgtccggcgttccatttggcatgacactacgaccaacacgatctcggttgtctcggcgcactccgtacagtagggatcgcctacctccttttgagacagagacccgcgctaccatactggaggatcatccgctgctgcccgaatgtaacactttgacaatgcacaacgtgagttacgtgcgaggtcttccctgcagtgtgggatttacgctgattcaggaatgggttgttccctgggatatggttctgacgcgggaggagcttgtaatcctgaggaagtgtatgcacgtgtgcctgtgttgtgccaacattgatatcatgacgagcatgatgatccatggttacggatcgcaggtgatagaggtctttcttccaaccagta

SEQ ID NO: 80 - DNA, 863 bp, synthetic construct
  misc_feature 1..863: note = fragment 14
  source 1..863: mol_type = other DNA
tagaggcaagggttgtttttattgactagaagacgatacgagtcctgggctctccactgtcattgttccagtcccggttccctgcagtgcatagccggcgggcaggttttggccagctggtttaggatggtggtggatggcgccatgtttaatcagaggtttatatggtaccgggaggtggtgaattacaacatgccaaaagaggtaatgtttatgtccagcgtgtttatgaggggtcgccacttaatctacctgcgcttgtggtatgatggccacgtgggttctgtggtccccgccatgagctttggatacagcgccttgcactgtgggattttgaacaatattgtggtgctgtgctgcagttactgtgctgatttaagtgagatcagggtgcgctgctgtgcccggaggacaaggcgtctcatgctgcgggcggtgcgaatcatcgctgaggagaccactgccatgttgtattcctgcaggacggagcggcggcggcagcagtttattcgcgcgctgctgcagcaccaccgccctatcctgatgcacgattatgactctacccccatgtaggcgtggacttccccttcgccgcccgttgagcaaccgcaagttggacagcagcctgtggctcagcagctggacagcgacatgaacttaagcgagctgcccggggagtttattaatatcactgatgagcgtttggctcgacaggaaaccgtgtggaatataacacctaagaatatgtctgttacccatgatatgatgctttttaaggccagccggggagaaaggactgtgtactctgtgtgttgggagggaggtggcaggagtcttcatagaggtctttcttccaaccagta

SEQ ID NO: 81 - DNA, 862 bp, synthetic construct
  misc_feature 1..862: note = fragment 15
  source 1..862: mol_type = other DNA
tagaggcaagggttgtttttattgactagaagacgagcaggttgaatactagggttctgtgagtttgattaaggtacggtgatcaatataagctatgtggtggtggggctatactactgaatgaaaaatgacttgaaattttctgcaattgaaaaataaacacgttgaaacataacatgcaacaggttcacgattctttattcctgggcaatgtaggagaaggtgtaagagttggtagcaaaagtttcagtggtgtattttccactttcccaggaccatgtaaaagacatagagtaagtgcttacctcgctagtttctgtggattcactagaatcgatgtaggatgttgcccctcctgacgcggtaggagaaggggagggtgccctgcatgtctgccgctgctcttgctcttgccgctgctgaggaggggggcgcatctgccgcagcaccggatgcatctgggaaaagcaaaaaaggggctcgtccctgtttccggaggaatttgcaagcggggtcttgcatgacggggaggcaaacccccgttcgccgcagtccggccggcccgagactcgaaccgggggtcctgcgactcaacccttggaaaataaccctccggctacagggagcgagccacttaatgctttcgctttccagcctaaccgcttacgccgcgcgcggccagtggccaaaaaagctagcgcagcagccgccgcgcctggaaggaagccaaaaggagcgctcccccgttgtctgacgtcgcacacctgggttcgacacgcgggcggtaaccgcatggatcacggcggacggccggatccggggttcgaacgagtcttcatagaggtctttcttccaaccagta

SEQ ID NO: 82 - DNA, 870 bp, synthetic construct
  misc_feature 1..870: note = fragment 16
  source 1..870: mol_type = other DNA
tagaggcaagggttgtttttattgactagaagacgagaaccccggtcgtccgccatgatacccttgcgaatttatccaccagaccacggaagagtgcccgcttacaggctctccttttgcacggtctagagcgtcaacgactgcgcacgcctcaccggccagagcgtcccgaccatggagcactttttgccgctgcgcaacatctggaaccgcgtccgcgactttccgcgcgcctccaccaccgccgccggcatcacctggatgtccaggtacatctacggattacgtcgacgtttaaaccatatgagcggccgctctagaactagtggatcccccggaagatcagaagttcctattccgaagttcctattctctagaaagtataggaacttctgatctgcgcagccgccatgccggggttttacgagattgtgattaaggtccccagcgaccttgacgagcatctgcccggcatttctgacagctttgtgaactgggtggccgagaaggaatgggagttgccgccagattctgacatggatctgaatctgattgagcaggcacccctgaccgtggccgagaagctgcagcgcgactttctgacggaatggcgccgtgtgagtaaggccccggaggcccttttctttgtgcaatttgagaagggagagagctacttccacatgcacgtgctcgtggaaaccaccggggtgaaatccatggttttgggacgtttcctgagtcagattcgcgaaaaactgattcagagaatttaccgcgggatcgagccgactttgccaaactggttcgcggtcacaaagaccagaaatggcgccggaggagtcttcatagaggtctttcttccaaccagta

SEQ ID NO: 83 - DNA, 875 bp, synthetic construct
  misc_feature 1..875: note = fragment 17
  source 1..875: mol_type = other DNA
tagaggcaagggttgtttttattgactacacctgcgatcggaggcgggaacaaggtggtggatgagtgctacatccccaattacttgctccccaaaacccagcctgagctccagtgggcgtggactaatatggaacagtatttaagcgcctgtttgaatctcacggagcgtaaacggttggtggcgcagcatctgacgcacgtgtcgcagacgcaggagcagaacaaagagaatcagaatcccaattctgatgcgccggtgatcagatcaaaaacttcagccaggtacatggagctggtcgggtggctcgtggacaaggggattacctcggagaagcagtggatccaggaggaccaggcctcatacatctccttcaatgcggcctccaactcgcggtcccaaatcaaggctgccttggacaatgcgggaaagattatgagcctgactaaaaccgcccccgactacctggtgggccagcagcccgtggaggacatttccagcaatcggatttataaaattttggaactaaacgggtacgatccccaatatgcggcttccgtctttctgggatgggccacgaaaaagttcggcaagaggaacaccatctggctgtttgggcctgcaactaccgggaagaccaacatcgcggaggccatagcccacactgtgcccttctacgggtgcgtaaactggaccaatgagaactttcccttcaacgactgtgtcgacaagatggtgatctggtgggaggaggggaagatgaccgccaaggtcgtggagtcggccaaagccattctcggaggaagcaaggtgcgcgtggaccagaaatgcaagtcctcgatcgcaggtgatagaggtctttcttccaaccagta

SEQ ID NO: 84 - DNA, 858 bp, synthetic construct
  misc_feature 1..858: note = fragment 18
  source 1..858: mol_type = other DNA
tagaggcaagggttgtttttattgactagaagacgacctcggcccagatagacccgactcccgtgatcgtcacctccaacaccaacatgtgcgccgtgattgacgggaactcaacgaccttcgaacaccagcagccgttgcaagaccggatgttcaaatttgaactcacccgccgtctggatcatgactttgggaaggtcaccaagcaggaagtcaaagactttttccggtgggcaaaggatcacgtggttgaggtggagcatgaattctacgtcaaaaagggtggagccaagaaaagacccgcccccagtgacgcagatataagtgagcccaaacgggtgcgcgagtcagttgcgcagccatcgacgtcagacgcggaagcttcgatcaactacgcagacaggtaccaaaacaaatgttctcgtcacgtgggcatgaatctgatgctgtttccctgcagacaatgcgagagaatgaatcagaattcaaatatctgcttcactcacggacagaaagactgtttagagtgctttcccgtgtcagaatctcaacccgtttctgtcgtcaaaaaggcgtatcagaaactgtgctacattcatcatatcatgggaaaggtgccagacgcttgcactgcctgcgatctggtcaatgtggatttggatgactgcatctttgaacaataaatgatttaaatcaggtatggctgccgatggttatcttccagattggctcgaggacactctctctgaaggaataagacagtggtggaagctcaaacctggcccaccaccaccaaagcccgcagagcggcataaggacgacagcgagtcttcatagaggtctttcttccaaccagta

SEQ ID NO: 85 - DNA, 875 bp, synthetic construct
  misc_feature 1..875: note = fragment 19
  source 1..875: mol_type = other DNA
tagaggcaagggttgtttttattgactacacctgcgatccagcaggggtcttgtgcttcctgggtacaagtacctcggacccttcaacggactcgacaagggagagccggtcaacgaggcagacgccgcggccctcgagcacgacaaagcctacgaccggcagctcgacagcggagacaacccgtacctcaagtacaaccacgccgacgcggagtttcaggagcgccttaaagaagatacgtcttttgggggcaacctcggacgagcagtcttccaggcgaaaaagagggttcttgaacctctgggcctggttgaggaacctgttaagacggctccgggaaaaaagaggccggtagagcactctcctgtggagccagactcctcctcgggaaccggaaaggcgggccagcagcctgcaagaaaaagattgaattttggtcagactggagacgcagactcagtacctgacccccagcctctcggacagccaccagcagccccctctggtctgggaactaatacgatggctacaggcagtggcgcaccaatggcagacaataacgagggcgccgacggagtgggtaattcctcgggaaattggcattgcgattccacatggatgggcgacagagtcatcaccaccagcacccgaacctgggccctgcccacctacaacaaccacctctacaaacaaatttccagccaatcaggagcctcgaacgacaatcactactttggctacagcaccccttgggggtattttgacttcaacagattccactgccacttttcaccacgtgactggcaaagactcatcaacaacaactggggattccgacgatcgcaggtgatagaggtctttcttccaaccagta

SEQ ID NO: 86 - DNA, 871 bp, synthetic construct
  misc_feature 1..871: note = fragment 20
  source 1..871: mol_type = other DNA
tagaggcaagggttgtttttattgactacacctgcgatccgacccaagagactcaacttcaagctctttaacattcaagtcaaagaggtcacgcagaatgacggtacgacgacgattgccaataaccttaccagcacggttcaggtgtttactgactcggagtaccagctcccgtacgtcctcggctcggcgcatcaaggatgcctcccgccgttcccagcagacgtcttcatggtgccacagtatggatacctcaccctgaacaacgggagtcaggcagtaggacgctcttcattttactgcctggagtactttccttctcagatgctgcgtaccggaaacaactttaccttcagctacacttttgaggacgttcctttccacagcagctacgctcacagccagagtctggaccgtctcatgaatcctctcatcgaccagtacctgtattacttgagcagaacaaacactccaagtggaaccaccacgcagtcaaggcttcagttttctcaggccggagcgagtgacattcgggaccagtctaggaactggcttcctggaccctgttaccgccagcagcgagtatcaaagacatctgcggataacaacaacagtgaatactcgtggactggagctaccaagtaccacctcaatggcagagactctctggtgaatccgggcccggccatggcaagccacaaggacgatgaagaaaagttttttcctcagagcggggttctcatctttgggaagcaaggctcagagaaaacaaatgtggacattgaaaaggtcatgattacagacgaagaggaaatcaggacaaccaatcccgtgggatcgcaggtgatagaggtctttcttccaaccagta

SEQ ID NO: 87 - DNA, 863 bp, synthetic construct
  misc_feature 1..863: note = fragment 21
  source 1..863: mol_type = other DNA
tagaggcaagggttgtttttattgactagaagacgagtggctacggagcagtatggttctgtatctaccaacctccagagaggcaacagacaagcagctaccgcagatgtcaacacacaaggcgttcttccaggcatggtctggcaggacagagatgtgtaccttcaggggcccatctgggcaaagattccacacacggacggacattttcacccctctcccctcatgggtggattcggacttaaacaccctcctccacagattctcatcaagaacaccccggtacctgcgaatccttcgaccaccttcagtgcggcaaagtttgcttccttcatcacacagtactccacgggacaggtcagcgtggagatcgagtgggagctgcagaaggaaaacagcaaacgctggaatcccgaaattcagtacacttccaactacaacaagtctgttaatgtggactttactgtggacactaatggcgtgtattcagagcctcgccccattggcaccagatacctgactcgtaatctgtaattgcttgttaatcaataaaccgtttaattcgtttcagttgaactttggtctctgcgtatttctttcttatctagtttccatggctactaaatggcccgcctggctgaccgcccaacgacccccgcccattgacgtcaataatgacgtatgttcccatagtaacgccaatagggactttccattgacgtcaatgggtggagtatttacggtaaactgcccacttggcagtacatcaagtgtatcatatgccaagtacgccccctattgacgtcaatgacggtaaatggcccgcctgggagtcttcatagaggtctttcttccaaccagta

SEQ ID NO: 88 - DNA, 862 bp, synthetic construct
  misc_feature 1..862: note = fragment 22
  source 1..862: mol_type = other DNA
tagaggcaagggttgtttttattgactagaagacgactggcattatgcccagtacatgaccttatgggactttcctacttggcagtacatctacgtattagtcatcgctattaccatggtgatgcggttttggcagtacatcaatgggcgtggatagcggtttgactcacggggatttccaagtctccaccccattgacgtcaatgggagtttgttttggcaccaaaatcaacgggactttccaaaatgtcgtaacaactccgccccattgacgcaaatgggcggtaggcgtgtacggtgggaggtctatataagcagagctggtttagtgaaccggatcctgccattgcatccttctctgcagactaagatggagttcctgaaccaagaccgcttgctggccaacctgtgaaactgggctcaaggtgaggggtgctatctgtgattgagggacatggttaatggaattgtctcacacagaaatcgcacccgtcaccttggcctacttatcaccaccccaaacagaggaacacgccttctccagccacagcctatggaagggccttcagctgctgtggccccgaggtaagcttgggggaggctaactgaaacacggaaggagacaataccggaaggaacccgcgctatgacggcaataaaaagacagaataaaacgcacggtgttgggtcgttgtagataagtagcatggcgggttaatcattaactacagcccggggtttaaacagcgggcggaggggtggagtcgtgacgtgaattacgtcatagggttagggaggtcctgtattagaggtcacgtgagtgttttgcgagtcttcatagaggtctttcttccaaccagta

SEQ ID NO: 89 - DNA, 875 bp, synthetic construct
  misc_feature 1..875: note = fragment 23
  source 1..875: mol_type = other DNA
tagaggcaagggttgtttttattgactacacctgcgatcttgcgacattttgcgacaccatgtggtctcgctgggggggggggcccgagtgagcacgcagggtctccattttgaagcgggaggtttgaacgagcgctggcgcgctccgtcgacgagctttaatgcggtagtttatcacagttaaattgctaacgcagtcaggcaccgtgtatgaaatctaacaatgcgctcatcgtcatcctcggcaccgtcaccctggatgctgtaggcataggcttggttatgccggtactgccgggcctcttgcgggatatcgtccattccgacagcatcgccagtcactatggcgtgctgctagcgctatatgcgttgatgcaatttctatgcgcacccgttctcggagcactgtccgaccgctttggccgccgcccagtcctgctcgcttcgctacttggagccactatcgactacgcgatcatggcgaccacacccgtcctgtggatcctctacgccggacgcatcgtggccggcatcaccggcgccacaggtgcggttgctggcgcctatatcgccgacatcaccgatggggaagatcgggctcgccacttcgggctcatgagcgcttgtttcggcgtgggtatggtggcaggccccgtggccgggggactgttgggcgccatctccttgcatgcaccattccttgcggcggcggtgctcaacggcctcaacctactactgggctgcttcctaatgcaggagtcgcataagggagagcgtcgaccgatgcccttgagagccttcaacccagtcagctccttccggtgggcgcggggcatgacgatcgcaggtgatagaggtctttcttccaaccagta

SEQ ID NO: 90 - DNA, 856 bp, synthetic construct
  misc_feature 1..856: note = fragment 24
  source 1..856: mol_type = other DNA
tagaggcaagggttgtttttattgactagaagacgatgactagatccacctgcacgtaaaaggccttcttggccgcccttcccggtcgatatgaacagcttatttacataattcacgttattggtagttataaatgaaattcctaatatcggttatgaagtgaaattgaatttctacttgatctttctctctatttttgtaaaataaaattaagaatatttaaatattcaatgattcatttttgcagaaatcggaggaagaagaatatatgaaaacatttaacatttctcaacaagatccccccatattgttgtataagtgatgaaatactgaatttaaaacttagtttatatgtggtaaaatgttttaatcaagtttaggaggaattaattatgaagtgtaatgaataatgaatgtaacagggttcaattaaaagagggaagcgtatcattaaccctataaactacgtctgccctcattattggagggtgaaatgtgaatacatcctattcacaatcgaatttacgacacaaccaaattttaatttggctttgcattttatctttttttagcgtattaaatgaaatggttttgaacgtctcattacctgatattgcaaatgattttaataaaccaccagcgagtacaaactgggtgaacacagcctttatgttaaccttttccattggaacagctgtatatggaaagctatctgatcaattaggcatcaaaaggttactcctatttggaattataataaattgtttcgggtcggtaattgggtttgttggccattctttcttttccttacttattatggctcgagtcttcatagaggtctttcttccaaccagta

SEQ ID NO: 91 - DNA, 881 bp, synthetic construct
  misc_feature 1..881: note = fragment 25
  source 1..881: mol_type = other DNA
tagaggcaagggttgtttttattgactacacctgcgatcgctcgttttattcaaggggctggtgcagctgcatttccagcactcgtaatggttgtagttgcgcgctatattccaaaggaaaataggggtaaagcatttggtcttattggatcgatagtagccatgggagaaggagtcggtccagcgattggtggaatgatagcccattatattcattggtcctatcttctactcattcctatgataacaattatcactgttccgtttcttatgaaattattaaagaaagaagtaaggataaaaggtcattttgatatcaaaggaattatactaatgtctgtaggcattgtattttttatgttgtttacaacatcatatagcatttcttttcttatcgttagcgtgctgtcattcctgatatttgtaaaacatatcaggaaagtaacagatccttttgttgatcccggattagggaaaaatataccttttatgattggagttctttgtgggggaattatatttggaacagtagcagggtttgtctctatggttccttatatgatgaaagatgttcaccagctaagtactgccgaaatcggaagtgtaattattttccctggaacaatgagtgtcattattttcggctacattggtgggatacttgttgatagaagaggtcctttatacgtgttaaacatcggagttacatttctttctgttagctttttaactgcttcctttcttttagaaacaacatcatggttcatgacaattataatcgtatttgttttaggtgggctttcgttcaccaaaacagttatatcaacaattgtttcaagtagcttgatcgcaggtgatagaggtctttcttccaaccagta

SEQ ID NO: 92 - DNA, 859 bp, synthetic construct
  misc_feature 1..859: note = fragment 26
  source 1..859: mol_type = other DNA
tagaggcaagggttgtttttattgactagaagacgagcttgaaacagcaggaagctggtgctggaatgagtttgcttaactttaccagctttttatcagagggaacaggtattgcaattgtaggtggtttattatccatacccttacttgatcaaaggttgttacctatggaagttgatcagtcaacttatctgtatagtaatttgttattacttttttcaggaatcattgtcattagttggctggttaccttgaatgtatataaacattctcaaagggatttctaaatcgttaagggatcaactttgggagagagttcaaaattgatcctttttttataacaggaattgggcatcaaataaaacgaaaggctcagtcgaaagactgggcctttcgttttatctgttgtttgtcggtgaacgctctcctgagtaggacaaatccgccgggagcggatttgaacgttgcgaagcaacggcccggagggtggcgggcaggacgcccgccataaactgccaggcatcaaattaagcagaaggccatcctgacggatggcctttttgcgtttctacaaactcttcctgtcgtcatatctacaattctacacagcccagtccagactattgaattgtatcacgtttttgatatcctaccaataacaaattgattggaggaatgcaaagtgaataatgaaccagtaaaacgtggtaagaagaacagatgggaattaaacctacctataatgacttatgtagtagctgatgattggattgataaactaggacacgaaacgtttactttatggttgaggttccatacttgggtagagtcttcatagaggtctttcttccaaccagta

SEQ ID NO: 93 - DNA, 879 bp, synthetic construct
  misc_feature 1..879: note = fragment 27
  source 1..879: mol_type = other DNA
tagaggcaagggttgtttttattgactacacctgcgatcggtagatagagaagatgaactccgagattatgatcgcatacctagaagttttgagaacatatataaaaagacactaggaatctcaaaaagtaagttttatagattgataaaacctttatgggaatatggattaatagacatcatagaatacgaagaatctaaccgtaattctactaaacctaaaaatataattgtttatgagtatcctttacacgaaatagaaagaaagtataaaccactagaaaaattaagagattgggataaagactataattccgtttctaaagaattaggtaaaacaggtggtagaccaaggaaaaaagatagtgaagaagaacccgaaaagaaacccgaagaagtaactaaaaagaaacgtaaatataagttaaaaagagttatccacaacggtttcaaaaatgaaacggtggagggtttcaaaaatgaaacggtggagggtttcaaaaatgaaacggtgaccgtttcaaaaataaaacccaataattattcaaatatctttaataacttatcaaatatttctactaatgtttcaaataatttattaattgatgatgatgaggaaatcgaaaatgaaccaactggtcgtacaataaataggtcattacttttttcacaagaagatattaaacaggcctatcaatttattaatagattttcagttatacagttacgtgaaaactttagctttgataaacactttgaagaacggttggtatgttatttatggaaagcagggatttctactttttacacgcacgaaatcagtaaaatgataaaaaaaatagcgatcgcaggtgatagaggtctttcttccaaccagta

SEQ ID NO: 94 - DNA, 865 bp, synthetic construct
  misc_feature 1..865: note = fragment 28
  source 1..865: mol_type = other DNA
tagaggcaagggttgtttttattgactagaagacgatagcagactatgaaaaatctaaaaaaggtagattaaacccaatacgtgaccgagccttatatatggtaaatggtcttgtaatgaatagagcttcttcccaaagtgaacatgctacttataaactaaaccaatataaaaaacagaaggaacaggaaaaacaacaacaggagcaacaaagatcaagagtaccgttctataattggttggaggaaagagaagaacaaaccgaaggtcaactacccaccacttaagcggccgcaagcttgaagagctcttctttcagaacgctcggttgccgccgggcgttttttatgagacgtctcggcctgtttggccattatactggcttaactatgcggcatcagagcagattgtactgagagtgcaccatatgcggtgtgaaataccgcacagatgcgtaaggagaaaataccgcatcaggcgctcttccgcttcctcgctcactgactcgctgcgctcggtcgttcggctgcggcgagcggtatcagctcactcaaaggcggtaatacggttatccacagaatcaggggataacgcaggaaagaacatgtgagcaaaaggccagcaaaaggccaggaaccgtaaaaaggccgcgttgctggcgtttttccataggctccgcccccctgacgagcatcacaaaaatcgacgctcaagtcagaggtggcgaaacccgacaggactataaagataccaggcgtttccccctggaagctccctcgtgcgctctcctgttccgaccctgccgcttaccggatacctgtccgcctttctcgagtcttcatagaggtctttcttccaaccagta

SEQ ID NO: 95 - DNA, 871 bp, synthetic construct
  misc_feature 1..871: note = fragment 29
  source 1..871: mol_type = other DNA
tagaggcaagggttgtttttattgactacacctgcgatctctcccttcgggaagcgtggcgctttctcatagctcacgctgtaggtatctcagttcggtgtaggtcgttcgctccaagctgggctgtgtgcacgaaccccccgttcagcccgaccgctgcgccttatccggtaactatcgtcttgagtccaacccggtaagacacgacttatcgccactggcagcagccactggtaacaggattagcagagcgaggtatgtaggcggtgctacagagttcttgaagtggtggcctaactacggctacactagaaggacagtatttggtatctgcgctctgctgaagccagttaccttcggaaaaagagttggtagctcttgatccggcaaacaaaccaccgctggtagcggtggtttttttgtttgcaagcagcagattacgcgcagaaaaaaaggatctcaagaagatcctttgatcttttctacggggtctgacgctcagtggaacgaaaactcacgttaagggattttggtcatgagattatcaaaaaggatcttcacctagatccttttaaattaaaaatgaagttttaaatcaatctaaagtatatatgagtaaacttggtctgacagttaccaatgcttaatcagtgaggcacctatctcagcgatctgtctatttcgttcatccatagttgcctgactccccgtcgtgtagataactacgatacgggagggcttaccatctggccccagtgctgcaatgataccgcgagacccacgctcaccggctccagatttatcagcaataaaccagccagccggaagggccgaggatcgcaggtgatagaggtctttcttccaaccagta

SEQ ID NO: 96 - DNA, 861 bp, synthetic construct
  misc_feature 1..861: note = fragment 30
  source 1..861: mol_type = other DNA
tagaggcaagggttgtttttattgactagaagacgacgagcgcagaagtggtcctgcaactttatccgcctccatccagtctattaattgttgccgggaagctagagtaagtagttcgccagttaatagtttgcgcaacgttgttgccattgctgcaggcatcgtggtgtcacgctcgtcgtttggtatggcttcattcagctccggttcccaacgatcaaggcgagttacatgatcccccatgttgtgcaaaaaagcggttagctccttcggtcctccgatcgttgtcagaagtaagttggccgcagtgttatcactcatggttatggcagcactgcataattctcttactgtcatgccatccgtaagatgcttttctgtgactggtgagtactcaaccaagtcattctgagaatagtgtatgcggcgaccgagttgctcttgcccggcgtcaacacgggataataccgcgccacatagcagaactttaaaagtgctcatcattggaaaacgttcttcggggcgaaaactctcaaggatcttaccgctgttgagatccagttcgatgtaacccactcgtgcacccaactgatcttcagcatcttttactttcaccagcgtttctgggtgagcaaaaacaggaaggcaaaatgccgcaaaaaagggaataagggcgacacggaaatgttgaatactcatactcttcctttttcaatattattgaagcatttatcagggttattgtctcatgagcggatacatatttgaatgtatttagaaaaataaacaaataggggttccgcggcgatcgccacatttccccgaaaagagtcttcatagaggtctttcttccaaccagta

SEQ ID NO: 97 - DNA, 168 bp, synthetic construct
  misc_feature 1..168: note = fragment 2 primer 1
  source 1..168: mol_type = other DNA
tagaggcaagggttgtttttattgactagaagacgagacgcaaatgggcggtaggcgtgtacggtgggaggtctatataagcagagctggtttagtggatatcgtatacgccaccatggtgagcaagggcgaggagctgttcaccggggtggtgcccatcctggtcga

SEQ ID NO: 98 - DNA, 165 bp, synthetic construct
  misc_feature 1..165: note = fragment 2 primer 2
  source 1..165: mol_type = other DNA
tggtcacgagggtgggccagggcacgggcagcttgccggtggtgcagatgaacttcagggtcagcttgccgtaggtggcatcgccctcgccctcgccggacacgctgaacttgtggccgtttacgtcgccgtccagctcgaccaggatgggcaccaccccggtga

SEQ ID NO: 99 - DNA, 168 bp, synthetic construct
  misc_feature 1..168: note = fragment 2 primer 3
  source 1..168: mol_type = other DNA
cccgtgccctggcccaccctcgtgaccaccctgacctacggcgtgcagtgcttcagccgctaccccgaccacatgaagcagcacgacttcttcaagtccgccatgcccgaaggctacgtccaggagcgcaccatcttcttcaaggacgacggcaactacaagacccgc

SEQ ID NO: 100 - DNA, 168 bp, synthetic construct
  misc_feature 1..168: note = fragment 2 primer 4
  source 1..168: mol_type = other DNA
ttgtcggccatgatatagacgttgtggctgttgtagttgtactccagcttgtgccccaggatgttgccgtcctccttgaagtcgatgcccttcagctcgatgcggttcaccagggtgtcgccctcgaacttcacctcggcgcgggtcttgtagttgccgtcgtccttg

SEQ ID NO: 101 - DNA, 168 bp, synthetic construct
  misc_feature 1..168: note = fragment 2 primer 5
  source 1..168: mol_type = other DNA
gccacaacgtctatatcatggccgacaagcagaagaacggcatcaaggtgaacttcaagatccgccacaacatcgaggacggcagcgtgcagctcgccgaccactaccagcagaacacccccatcggcgacggccccgtgctgctgcccgacaaccactacctgagca

SEQ ID NO: 102 - DNA, 168 bp, synthetic construct
  misc_feature 1..168: note = fragment 2 primer 6
  source 1..168: mol_type = other DNA
tactggttggaagaaagacctctatgaagactccttgtacagctcgtccatgccgagagtgatcccggcggcggtcacgaactccagcaggaccatgtgatcgcgcttctcgttggggtctttgctcagggcggactgggtgctcaggtagtggttgtcgggcagcag

SEQ ID NO: 103 - DNA, 171 bp, synthetic construct
  misc_feature 1..171: note = fragment 3 primer 1
  source 1..171: mol_type = other DNA
tagaggcaagggttgtttttattgactacacctgcgatccaagtaagtataccgataatcaacctctggattacaaaatttgtgaaagattgactggtattcttaactatgttgctccttttacgctatgtggatacgctgctttaatgcctttgtatcatgctattgctt

SEQ ID NO: 104 - DNA, 171 bp, synthetic construct
  misc_feature 1..171: note = fragment 3 primer 2
  source 1..171: mol_type = other DNA
tggcaatgccccaaccagtgggggttgcgtcagcaaacacagtgcacaccacgccacgttgcctgacaacgggccacaactcctcataaagagacagcaaccaggatttatacaaggaggagaaaatgaaagccatacgggaagcaatagcatgatacaaaggcattaaag

SEQ ID NO: 105 - DNA, 167 bp, synthetic construct
  misc_feature 1..167: note = fragment 3 primer 3
  source 1..167: mol_type = other DNA
acgcaacccccactggttggggcattgccaccacctgtcagctcctttccgggactttcgctttccccctccctattgccacggcggaactcatcgccgcctgccttgcccgctgctggacaggggctcggctgttgggcactgacaattccgtggtgttgtcgggg

SEQ ID NO: 106 - DNA, 171 bp, synthetic construct
  misc_feature 1..171: note = fragment 3 primer 4
  source 1..171: mol_type = other DNA
cggaagaggccgcagagccggcagcaggccgcgggaaggaaggtccgctggattgagggccgaagggacgtagcagaaggacgtcccgcgcagaatccaggtggcaacacaggcgagcagccatggaaaggacgtcagcttccccgacaacaccacggaattgtcagtgcc

SEQ ID NO: 107 - DNA, 171 bp, synthetic construct
  misc_feature 1..171: note = fragment 3 primer 5
  source 1..171: mol_type = other DNA
ggcctgctgccggctctgcggcctcttccgcgtcttcgccttcgccctcagacgagtcggatctccctttgggccgcctccccgcatcggttaattaaacgggtggcatccctgtgacccctccccagtgcctctcctggccctggaagttgccactccagtgcccaccag

SEQ ID NO: 108 - DNA, 171 bp, synthetic construct
  misc_feature 1..171: note = fragment 3 primer 6
  source 1..171: mol_type = other DNA
tactggttggaagaaagacctctatcacctgcgatcttcccaacttgccccttgctccataccacccccctccaccccataatattatagaaggacacctagtcagacaaaatgatgcaacttaattttattaggacaaggctggtgggcactggagtggcaacttccagg

SEQ ID NO: 109 - DNA, 171 bp, synthetic construct
  misc_feature 1..171: note = fragment 4 primer 1
  source 1..171: mol_type = other DNA
tagaggcaagggttgtttttattgactacacctgcgatcggaagacaacctgtagggcctgcggggtctattgggaaccaagctggagtgcagtggcacaatcttggctcactgcaatctccgcctcctgggttcaagcgattctcctgcctcagcctcccgagttgttgg

SEQ ID NO: 110 - DNA, 171 bp, synthetic construct
  misc_feature 1..171: note = fragment 4 primer 2
  source 1..171: mol_type = other DNA
gtaatcccagcaatttgggaggccaaggtgggtagatcacctgagattaggagttggagaccagcctggccaatatggtgaaaccccgtctctaccaaaaaaacaaaaattagctgagcctggtcatgcatgcctggaatcccaacaactcgggaggctgaggcaggagaa

SEQ ID NO: 111 - DNA, 169 bp, synthetic construct
  misc_feature 1..169: note = fragment 4 primer 3
  source 1..169: mol_type = other DNA
caccttggcctcccaaattgctgggattacaggcgtgaaccactgctcccttccctgtccttatcgatagatctaggaacccctagtgatggagttggccactccctctctgcgcgctcgctcgctcactgaggccgggcgaccaaaggtcgcccgacgcccgggcttt

SEQ ID NO: 112 - DNA, 171 bp, synthetic construct
  misc_feature 1..171: note = fragment 4 primer 4
  source 1..171: mol_type = other DNA
ccaggaagctgtagagctgttcctggttgcgacgcagggtgggctgtacctggggactgttaagcatggagttgggtacccctcgaggggatctgcctgcaggcagctgcgcgctcgctcgctcactgaggccgcccgggcaaagcccgggcgtcgggcgacctttggtcg

SEQ ID NO: 113 - DNA, 171 bp, synthetic construct
  misc_feature 1..171: note = fragment 4 primer 5
  source 1..171: mol_type = other DNA
gcaaccaggaacagctctacagcttcctggagcgccactcgccctacttccgcagccacagtgcgcagattaggagcgccacttctttttgtcacttgaaaaacatgtaaaaataatgtactaggagacactttcaataaaggcaaatgtttttatttgtacactctcggg

SEQ ID NO: 114 - DNA, 171 bp, synthetic construct
  misc_feature 1..171: note = fragment 4 primer 6
  source 1..171: mol_type = other DNA
tactggttggaagaaagacctctatcacctgcgatccaccagtatcgcaacgtgtccctgccagtggcgcatagcgatgcgcggcagaacccctttgatttttaaacggcgcagacggcaagggtggggggtaaataatcacccgagagtgtacaaataaaaacatttgcc

SEQ ID NO: 115 - DNA, 169 bp, synthetic construct
  misc_feature 1..169: note = fragment 22 primer 1
  source 1..169: mol_type = other DNA
tagaggcaagggttgtttttattgactagaagacgactggcattatgcccagtacatgaccttatgggactttcctacttggcagtacatctacgtattagtcatcgctattaccatggtgatgcggttttggcagtacatcaatgggcgtggatagcggtttgactca

SEQ ID NO: 116 - DNA, 169 bp, synthetic construct
  misc_feature 1..169: note = fragment 22 primer 2
  source 1..169: mol_type = other DNA
agacctcccaccgtacacgcctaccgcccatttgcgtcaatggggcggagttgttacgacattttggaaagtcccgttgattttggtgccaaaacaaactcccattgacgtcaatggggtggagacttggaaatccccgtgagtcaaaccgctatccacgcccattgat

SEQ ID NO: 117 - DNA, 167 bp, synthetic construct
  misc_feature 1..167: note = fragment 22 primer 3
  source 1..167: mol_type = other DNA
tgggcggtaggcgtgtacggtgggaggtctatataagcagagctggtttagtgaaccggatcctgccattgcatccttctctgcagactaagatggagttcctgaaccaagaccgcttgctggccaacctgtgaaactgggctcaaggtgaggggtgctatctgtga

SEQ ID NO: 118 - DNA, 169 bp, synthetic construct
  misc_feature 1..169: note = fragment 22 primer 4
  source 1..169: mol_type = other DNA
tcggggccacagcagctgaaggcccttccataggctgtggctggagaaggcgtgttcctctgtttggggtggtgataagtaggccaaggtgacgggtgcgatttctgtgtgagacaattccattaaccatgtccctcaatcacagatagcacccctcaccttgagccca

SEQ ID NO: 119 - DNA, 169 bp, synthetic construct
  misc_feature 1..169: note = fragment 22 primer 5
  source 1..169: mol_type = other DNA
tggaagggccttcagctgctgtggccccgaggtaagcttgggggaggctaactgaaacacggaaggagacaataccggaaggaacccgcgctatgacggcaataaaaagacagaataaaacgcacggtgttgggtcgttgtagataagtagcatggcgggttaatcatt

SEQ ID NO: 120 - DNA, 169 bp, synthetic construct
  misc_feature 1..169: note = fragment 22 primer 6
  source 1..169: mol_type = other DNA
tactggttggaagaaagacctctatgaagactcgcaaaacactcacgtgacctctaatacaggacctccctaaccctatgacgtaattcacgtcacgactccacccctccgcccgctgtttaaaccccgggctgtagttaatgattaacccgccatgctacttatctac

SEQ ID NO: 121 - DNA, 171 bp, synthetic construct
  misc_feature 1..171: note = fragment 23 primer 1
  source 1..171: mol_type = other DNA
tagaggcaagggttgtttttattgactacacctgcgatcttgcgacattttgcgacaccatgtggtctcgctgggggggggggcccgagtgagcacgcagggtctccattttgaagcgggaggtttgaacgagcgctggcgcgctccgtcgacgagctttaatgcggtagt

SEQ ID NO: 122 - DNA, 171 bp, synthetic construct
  misc_feature 1..171: note = fragment 23 primer 2
  source 1..171: mol_type = other DNA
atcccgcaagaggcccggcagtaccggcataaccaagcctatgcctacagcatccagggtgacggtgccgaggatgacgatgagcgcattgttagatttcatacacggtgcctgactgcgttagcaatttaactgtgataaactaccgcattaaagctcgtcgacggagcg

SEQ ID NO: 123 - DNA, 170 bp, synthetic construct
  misc_feature 1..170: note = fragment 23 primer 3
  source 1..170: mol_type = other DNA
atgccggtactgccgggcctcttgcgggatatcgtccattccgacagcatcgccagtcactatggcgtgctgctagcgctatatgcgttgatgcaatttctatgcgcacccgttctcggagcactgtccgaccgctttggccgccgcccagtcctgctcgcttcgctact

SEQ ID NO: 124 - DNA, 171 bp, synthetic construct
  misc_feature 1..171: note = fragment 23 primer 4
  source 1..171: mol_type = other DNA
tcttccccatcggtgatgtcggcgatataggcgccagcaaccgcacctgtggcgccggtgatgccggccacgatgcgtccggcgtagaggatccacaggacgggtgtggtcgccatgatcgcgtagtcgatagtggctccaagtagcgaagcgagcaggactgggcggcgg

SEQ ID NO: 125 - DNA, 171 bp, synthetic construct
  misc_feature 1..171: note = fragment 23 primer 5
  source 1..171: mol_type = other DNA
ctatatcgccgacatcaccgatggggaagatcgggctcgccacttcgggctcatgagcgcttgtttcggcgtgggtatggtggcaggccccgtggccgggggactgttgggcgccatctccttgcatgcaccattccttgcggcggcggtgctcaacggcctcaacctact

SEQ ID NO: 126 - DNA, 171 bp, synthetic construct
  misc_feature 1..171: note = fragment 23 primer 6
  source 1..171: mol_type = other DNA
tactggttggaagaaagacctctatcacctgcgatcgtcatgccccgcgcccaccggaaggagctgactgggttgaaggctctcaagggcatcggtcgacgctctcccttatgcgactcctgcattaggaagcagcccagtagtaggttgaggccgttgagcaccgccgcc

SEQ ID NO: 127 - DNA, 170 bp, synthetic construct
  misc_feature 1..170: note = fragment 28 primer 1
  source 1..170: mol_type = other DNA
tagaggcaagggttgtttttattgactagaagacgatagcagactatgaaaaatctaaaaaaggtagattaaacccaatacgtgaccgagccttatatatggtaaatggtcttgtaatgaatagagcttcttcccaaagtgaacatgctacttataaactaaaccaatat

SEQ ID NO: 128 - DNA, 170 bp, synthetic construct
  misc_feature 1..170: note = fragment 28 primer 2
  source 1..170: mol_type = other DNA
gagctcttcaagcttgcggccgcttaagtggtgggtagttgaccttcggtttgttcttctctttcctccaaccaattatagaacggtactcttgatctttgttgctcctgttgttgtttttcctgttccttctgttttttatattggtttagtttataagtagcatgttc

SEQ ID NO: 129 - DNA, 165 bp, synthetic construct
  misc_feature 1..165: note = fragment 28 primer 3
  source 1..165: mol_type = other DNA
cacttaagcggccgcaagcttgaagagctcttctttcagaacgctcggttgccgccgggcgttttttatgagacgtctcggcctgtttggccattatactggcttaactatgcggcatcagagcagattgtactgagagtgcaccatatgcggtgtgaaataccg

SEQ ID NO: 130 - DNA, 170 bp, synthetic construct
  misc_feature 1..170: note = fragment 28 primer 4
  source 1..170: mol_type = other DNA
cctgattctgtggataaccgtattaccgcctttgagtgagctgataccgctcgccgcagccgaacgaccgagcgcagcgagtcagtgagcgaggaagcggaagagcgcctgatgcggtattttctccttacgcatctgtgcggtatttcacaccgcatatggtgcactct

SEQ ID NO: 131 - DNA, 170 bp, synthetic construct
  misc_feature 1..170: note = fragment 28 primer 5
  source 1..170: mol_type = other DNA
ggcggtaatacggttatccacagaatcaggggataacgcaggaaagaacatgtgagcaaaaggccagcaaaaggccaggaaccgtaaaaaggccgcgttgctggcgtttttccataggctccgcccccctgacgagcatcacaaaaatcgacgctcaagtcagaggtggc

SEQ ID NO: 132 - DNA, 170 bp, synthetic construct
  misc_feature 1..170: note = fragment 28 primer 6
  source 1..170: mol_type = other DNA
tactggttggaagaaagacctctatgaagactcgagaaaggcggacaggtatccggtaagcggcagggtcggaacaggagagcgcacgagggagcttccagggggaaacgcctggtatctttatagtcctgtcgggtttcgccacctctgacttgagcgtcgatttttgt

SEQ ID NO: 133 - DNA, 165 bp, synthetic construct
  misc_feature 1..165: note = fragment 30 primer 1
  source 1..165: mol_type = other DNA
tagaggcaagggttgtttttattgactagaagacgacgagcgcagaagtggtcctgcaactttatccgcctccatccagtctattaattgttgccgggaagctagagtaagtagttcgccagttaatagtttgcgcaacgttgttgccattgctgcaggcatcgt

SEQ ID NO: 134 - DNA, 168 bp, synthetic construct
  misc_feature 1..168: note = fragment 30 primer 2
  source 1..168: mol_type = other DNA
cggccaacttacttctgacaacgatcggaggaccgaaggagctaaccgcttttttgcacaacatgggggatcatgtaactcgccttgatcgttgggaaccggagctgaatgaagccataccaaacgacgagcgtgacaccacgatgcctgcagcaatggcaacaacgt

SEQ ID NO: 135 - DNA, 165 bp, synthetic construct
  misc_feature 1..165: note = fragment 30 primer 3
  source 1..165: mol_type = other DNA
ccgatcgttgtcagaagtaagttggccgcagtgttatcactcatggttatggcagcactgcataattctcttactgtcatgccatccgtaagatgcttttctgtgactggtgagtactcaaccaagtcattctgagaatagtgtatgcggcgaccgagttgctct

SEQ ID NO: 136 - DNA, 168 bp, synthetic construct
  misc_feature 1..168: note = fragment 30 primer 4
  source 1..168: mol_type = other DNA
gcacgagtgggttacatcgaactggatctcaacagcggtaagatccttgagagttttcgccccgaagaacgttttccaatgatgagcacttttaaagttctgctatgtggcgcggtattatcccgtgttgacgccgggcaagagcaactcggtcgccgcatacactat

SEQ ID NO: 137 - DNA, 167 bp, synthetic construct
  misc_feature 1..167: note = fragment 30 primer 5
  source 1..167: mol_type = other DNA
gatccagttcgatgtaacccactcgtgcacccaactgatcttcagcatcttttactttcaccagcgtttctgggtgagcaaaaacaggaaggcaaaatgccgcaaaaaagggaataagggcgacacggaaatgttgaatactcatactcttcctttttcaatattat

SEQ ID NO: 138 - DNA, 168 bp, synthetic construct
  misc_feature 1..168: note = fragment 30 primer 6
  source 1..168: mol_type = other DNA
tactggttggaagaaagacctctatgaagactcttttcggggaaatgtggcgatcgccgcggaacccctatttgtttatttttctaaatacattcaaatatgtatccgctcatgagacaataaccctgataaatgcttcaataatattgaaaaaggaagagtatgagt

SEQ ID NO: 139 - DNA, 36 bp, synthetic construct
  misc_feature 1..36: note = fragment 1-F
  source 1..36: mol_type = other DNA
tagcacctgcgatcaaaagtgccacctgacgtctaa

SEQ ID NO: 140 - DNA, 35 bp, synthetic construct
  misc_feature 1..35: note = fragment 5-F
  source 1..35: mol_type = other DNA
taggaagacgaggtgtttagtgctccacttaaact

SEQ ID NO: 141 - DNA, 38 bp, synthetic construct
  misc_feature 1..38: note = fragment 6-F
  source 1..38: mol_type = other DNA
tagcacctgcgatccatcatcgtcacaaaggtcttgtt

SEQ ID NO: 142 - DNA, 30 bp, synthetic construct
  misc_feature 1..30: note = fragment 7-F
  source 1..30: mol_type = other DNA
tagcacctgcgatccctaaccgcccccttt

SEQ ID NO: 143 - DNA, 33 bp, synthetic construct
  misc_feature 1..33: note = fragment 8-F
  source 1..33: mol_type = other DNA
taggaagacgaccaaggttatgagcacagtcat

SEQ ID NO: 144 - DNA, 34 bp, synthetic construct
  misc_feature 1..34: note = fragment 9-F
  source 1..34: mol_type = other DNA
tagcacctgcgatccttctgcagctagccaacta

SEQ ID NO: 145 - DNA, 31 bp, synthetic construct
  misc_feature 1..31: note = fragment 10-F
  source 1..31: mol_type = other DNA
tagcacctgcgatcgacccaaccgtagatgg

SEQ ID NO: 146 - DNA, 27 bp, synthetic construct
  misc_feature 1..27: note = fragment 11-F
  source 1..27: mol_type = other DNA
taggaagacgactacatgagcgcggga

SEQ ID NO: 147 - DNA, 34 bp, synthetic construct
  misc_feature 1..34: note = fragment 12-F
  source 1..34: mol_type = other DNA
taggaagacgacctgatgtgtttaccgagtctta

SEQ ID NO: 148 - DNA, 31 bp, synthetic construct
  misc_feature 1..31: note = fragment 13-F
  source 1..31: mol_type = other DNA
tagcacctgcgatcgtccacttggacgtgag

SEQ ID NO: 149 - DNA, 28 bp, synthetic construct
  misc_feature 1..28: note = fragment 14-F
  source 1..28: mol_type = other DNA
taggaagacgatacgagtcctgggctct

SEQ ID NO: 150 - DNA, 33 bp, synthetic construct
  misc_feature 1..33: note = fragment 15-F
  source 1..33: mol_type = other DNA
taggaagacgagcaggttgaatactagggttct

SEQ ID NO: 151 - DNA, 25 bp, synthetic construct
  misc_feature 1..25: note = fragment 16-F
  source 1..25: mol_type = other DNA
taggaagacgagaaccccggtcgtc

SEQ ID NO: 152 - DNA, 29 bp, synthetic construct
  misc_feature 1..29: note = fragment 17-F
  source 1..29: mol_type = other DNA
tagcacctgcgatcggaggcgggaacaag

SEQ ID NO: 153 - DNA, 27 bp, synthetic construct
  misc_feature 1..27: note = fragment 18-F
  source 1..27: mol_type = other DNA
taggaagacgacctcggcccagataga

SEQ ID NO: 154 - DNA, 30 bp, synthetic construct
  misc_feature 1..30: note = fragment 19-F
  source 1..30: mol_type = other DNA
tagcacctgcgatccagcaggggtcttgtg

SEQ ID NO: 155 - DNA, 34 bp, synthetic construct
  misc_feature 1..34: note = fragment 20-F
  source 1..34: mol_type = other DNA
tagcacctgcgatccgacccaagagactcaactt

SEQ ID NO: 156 - DNA, 29 bp, synthetic construct
  misc_feature 1..29: note = fragment 21-F
  source 1..29: mol_type = other DNA
taggaagacgagtggctacggagcagtat

SEQ ID NO: 157 - DNA, 30 bp, synthetic construct
  misc_feature 1..30: note = fragment 24-F
  source 1..30: mol_type = other DNA
taggaagacgatgactagatccacctgcac

SEQ ID NO: 158 - DNA, 35 bp, synthetic construct
  misc_feature 1..35: note = fragment 25-F
  source 1..35: mol_type = other DNA
tagcacctgcgatcgctcgttttattcaaggggct

SEQ ID NO: 159 - DNA, 31 bp, synthetic construct
  misc_feature 1..31: note = fragment 26-F
  source 1..31: mol_type = other DNA
taggaagacgagcttgaaacagcaggaagct

SEQ ID NO: 160 - DNA, 37 bp, synthetic construct
  misc_feature 1..37: note = fragment 27-F
  source 1..37: mol_type = other DNA
tagcacctgcgatcggtagatagagaagatgaactcc

SEQ ID NO: 161 - DNA, 30 bp, synthetic construct
  misc_feature 1..30: note = fragment 29-F
  source 1..30: mol_type = other DNA
tagcacctgcgatctctcccttcgggaagc

SEQ ID NO: 162 - DNA, 29 bp, synthetic construct
  misc_feature 1..29: note = fragment 1-R
  source 1..29: mol_type = other DNA
tagcacctgcgatccgtcaatggggcgga

SEQ ID NO: 163 - DNA, 27 bp, synthetic construct
  misc_feature 1..27: note = fragment 5-R
  source 1..27: mol_type = other DNA
taggaagactcgatggggcgattcctg

SEQ ID NO: 164 - DNA, 32 bp, synthetic construct
  misc_feature 1..32: note = fragment 6-R
  source 1..32: mol_type = other DNA
tagcacctgcgatctaggctgtcctccttctc

SEQ ID NO: 165 - DNA, 33 bp, synthetic construct
  misc_feature 1..33: note = fragment 7-R
  source 1..33: mol_type = other DNA
tagcacctgcgatcttggggggtaggttaagtg

SEQ ID NO: 166 - DNA, 28 bp, synthetic construct
  misc_feature 1..28: note = fragment 8-R
  source 1..28: mol_type = other DNA
taggaagactcgaaggtagcagtgaccc

SEQ ID NO: 167 - DNA, 28 bp, synthetic construct
  misc_feature 1..28: note = fragment 9-R
  source 1..28: mol_type = other DNA
tagcacctgcgatcggtcggcgaacagg

SEQ ID NO: 168 - DNA, 40 bp, synthetic construct
  misc_feature 1..40: note = fragment 10-R
  source 1..40: mol_type = other DNA
tagcacctgcgatcgtagtttattcgggttgagtagtctt

SEQ ID NO: 169 - DNA, 32 bp, synthetic construct
  misc_feature 1..32: note = fragment 11-R
  source 1..32: mol_type = other DNA
taggaagactccaggttggttaacatcggtca

SEQ ID NO: 170 - DNA, 32 bp, synthetic construct
  misc_feature 1..32: note = fragment 12-R
  source 1..32: mol_type = other DNA
taggaagactcggacgtaaaggctaaaccctt

SEQ ID NO: 171 - DNA, 36 bp, synthetic construct
  misc_feature 1..36: note = fragment 13-R
  source 1..36: mol_type = other DNA
tagcacctgcgatccgtaaccatggatcatcatgct

SEQ ID NO: 172 - DNA, 25 bp, synthetic construct
  misc_feature 1..25: note = fragment 14-R
  source 1..25: mol_type = other DNA
taggaagactcctgccacctccctc

SEQ ID NO: 173 - DNA, 27 bp, synthetic construct
  misc_feature 1..27: note = fragment 15-R
  source 1..27: mol_type = other DNA
taggaagactcgttcgaaccccggatc

SEQ ID NO: 174 - DNA, 27 bp, synthetic construct
  misc_feature 1..27: note = fragment 16-R
  source 1..27: mol_type = other DNA
taggaagactcctccggcgccatttct

SEQ ID NO: 175 - DNA, 34 bp, synthetic construct
  misc_feature 1..34: note = fragment 17-R
  source 1..34: mol_type = other DNA
tagcacctgcgatcgaggacttgcatttctggtc

SEQ ID NO: 176 - DNA, 28 bp, synthetic construct
  misc_feature 1..28: note = fragment 18-R
  source 1..28: mol_type = other DNA
taggaagactcgctgtcgtccttatgcc

SEQ ID NO: 177 - DNA, 33 bp, synthetic construct
  misc_feature 1..33: note = fragment 19-R
  source 1..33: mol_type = other DNA
tagcacctgcgatcgtcggaatccccagttgtt

SEQ ID NO: 178 - DNA, 31 bp, synthetic construct
  misc_feature 1..31: note = fragment 20-R
  source 1..31: mol_type = other DNA
tagcacctgcgatcccacgggattggttgtc

SEQ ID NO: 179 - DNA, 25 bp, synthetic construct
  misc_feature 1..25: note = fragment 21-R
  source 1..25: mol_type = other DNA
taggaagactcccaggcgggccatt

SEQ ID NO: 180 - DNA, 42 bp, synthetic construct
  misc_feature 1..42: note = fragment 24-R
  source 1..42: mol_type = other DNA
taggaagactcgagccataataagtaaggaaaagaaagaatg

SEQ ID NO: 181 - DNA, 50 bp, synthetic construct
  misc_feature 1..50: note = fragment 25-R
  source 1..50: mol_type = other DNA
tagcacctgcgatcaagctacttgaaacaattgttgatataactgttttg

SEQ ID NO: 182 - DNA, 33 bp, synthetic construct
  misc_feature 1..33: note = fragment 26-R
  source 1..33: mol_type = other DNA
taggaagactctacccaagtatggaacctcaac

SEQ ID NO: 183 - DNA, 49 bp, synthetic construct
  misc_feature 1..49: note = fragment 27-R
  source 1..49: mol_type = other DNA
tagcacctgcgatcgctattttttttatcattttactgatttcgtgcgt

SEQ ID NO: 184 - DNA, 27 bp, synthetic construct
  misc_feature 1..27: note = fragment 29-R
  source 1..27: mol_type = other DNA
tagcacctgcgatcctcggcccttccg

SEQ ID NO: 185 - DNA, 20 bp, synthetic construct
  misc_feature 1..20: note = CMV primer 1
  source 1..20: mol_type = other DNA
catcaatgggcgtggatagc

SEQ ID NO: 186 - DNA, 24 bp, synthetic construct
  misc_feature 1..24: note = CMV primer 2
  source 1..24: mol_type = other DNA
ggagttgttacgacattttggaaa

SEQ ID NO: 187 - DNA, 20 bp, synthetic construct
  misc_feature 1..20: note = EGFP-WPRE primer 1
  source 1..20: mol_type = other DNA
gagctggtttagtggatatc

SEQ ID NO: 188 - DNA, 23 bp, synthetic construct
  misc_feature 1..23: note = EGFP-WPRE primer 2
  source 1..23: mol_type = other DNA
cagggatgccacccgtttaatta